European Patent Specification EP 3 597 183 B1, published June 28, 2023. Title: Composition for suppressing growth of microorganism equiping menaquinone biosynthetic pathway via futalosine or futalosine derivative. Applicant: Nitto Pharmaceutical Industries, Ltd. The sequence listing filed with the application follows.

SEQUENCE LISTING (10 sequences)

SEQ ID NO: 1 - DNA, 20 bp, Artificial Sequence
  primer
aagtcgaacgatgaagccta

SEQ ID NO: 2 - DNA, 22 bp, Artificial Sequence
  primer
atttggtattaatcaccatttc

SEQ ID NO: 3 - DNA, 25 bp, Artificial Sequence
  primer
tcacccacactgtgcccatctacga

SEQ ID NO: 4 - DNA, 24 bp, Artificial Sequence
  primer
ggatgccacaggattccataccca

SEQ ID NO: 5 - DNA, 18 bp, Artificial Sequence
  primer
agtgactagcctggactt

SEQ ID NO: 6 - DNA, 18 bp, Artificial Sequence
  primer
actgactgacaccatctg

SEQ ID NO: 7 - DNA, 18 bp, Artificial Sequence
  primer
caggaagagtttggtcaa

SEQ ID NO: 8 - DNA, 19 bp, Artificial Sequence
  primer
ggttcacagtcgtagatat

SEQ ID NO: 9 - DNA, 20 bp, Artificial Sequence
  primer
tgtgtccgtcgtggatctga

SEQ ID NO: 10 - DNA, 21 bp, Artificial Sequence
  primer
ttgctgttgaagtcgcaggag